European Patent Application EP 4 556 492 A1, published May 21, 2025. Title: TREATMENT OF CARDIOVASCULAR DISEASES USING ANTI-HUMAN GPVI ANTIBODIES IN SUBPOPULATIONS OF SUBJECTS. Applicant: ACTICOR BIOTECH. The sequence listing filed with the application follows.

SEQUENCE LISTING (21 sequences)

SEQ ID NO: 1 - protein, 10 aa, synthetic construct
  REGION 1..10: note = VH-CDR1
GYTFTSYNMH

SEQ ID NO: 2 - protein, 17 aa, synthetic construct
  REGION 1..17: note = VH-CDR2
GIYPGNGDTSYNQKFQG

SEQ ID NO: 3 - protein, 11 aa, synthetic construct
  REGION 1..11: note = VH-CDR3
GTVVGDWYFDV

SEQ ID NO: 4 - protein, 16 aa, synthetic construct
  REGION 1..16: note = VL-CDR1
RSSQSLENSNGNTYLN

SEQ ID NO: 5 - protein, 7 aa, synthetic construct
  REGION 1..7: note = VL-CDR2
RVSNRFS

SEQ ID NO: 6 - protein, 9 aa, synthetic construct
  REGION 1..9: note = VL-CDR3
LQLTHVPWT

SEQ ID NO: 7 - protein, 120 aa, synthetic construct
  REGION 1..120: note = heavy chain variable region
QVQLVQSGAEVKKPGASVKVSCKASGYTFTSYNMHWVRQAPGQGLEWMGGIYPGNGDTSYNQKFQGRVTMTRDTSTSTVYMELSSLRSEDTAVYYCARGTVVGDWYFDVWGQGTLVTVSS

SEQ ID NO: 8 - protein, 113 aa, synthetic construct
  REGION 1..113: note = light chain variable region
DIQMTQSPSSLSASVGDRVTITCRSSQSLENSNGNTYLNWYQQKPGKAPKLLIYRVSNRFSGVPSRFSGSGSGTDFTFTISSLQPEDIATYYCLQLTHVPWTFGQGTKVEITR

SEQ ID NO: 9 - protein, 113 aa, synthetic construct
  REGION 1..113: note = light chain variable region
DIQMTQSPSSLSASVGDRVTITCSASQSLENSNGNTYLNWYQQKPGKAPKLLIYRVSNRFSGVPSRFSGSGSGTDFTLTISSLQPEDFATYYCLQLTHVPWTFGQGTKVEIKR

SEQ ID NO: 10 - DNA, 360 bp, synthetic construct
  source 1..360: mol_type = other DNA
  misc_feature 1..360: note = heavy chain variable region
caggttcagctggttcagtcaggggctgaggtgaagaagcctggagcctcagtgaaggtgtcctgcaaggcttctggctacacatttaccagttacaatatgcactgggtaagacaggctcctggacagggcctggaatggatgggaggtatttatccaggaaatggtgatacttcctacaatcagaagttccagggccgagttactatgactcgggacacttccacctctacagtgtacatggagctcagcagcctgagatctgaggacaccgcggtctattactgtgcaagaggcaccgtggtcggcgactggtacttcgatgtgtggggccaaggcaccctggtcaccgtgagcagt

SEQ ID NO: 11 - DNA, 339 bp, synthetic construct
  source 1..339: mol_type = other DNA
  misc_feature 1..339: note = light chain variable region
gacatccagatgacccagagcccaagcagcctgagcgccagcgtgggtgacagagtgaccatcacctgtagaagtagtcagagccttgagaacagcaacggaaacacctacctgaattggtaccagcagaagccaggtaaggctccaaagctgctgatctacagagtttccaaccgattctctggtgtgccaagcagattcagcggtagcggtagcggtaccgacttcaccttcaccatcagcagcctccagccagaggacatcgccacctactactgcctccagctgactcatgtcccatggaccttcggtcagggcaccaaggtggagatcacccgg

SEQ ID NO: 12 - DNA, 339 bp, synthetic construct
  source 1..339: mol_type = other DNA
  misc_feature 1..339: note = light chain variable region
gacatccagatgacccagagcccaagcagcctgagcgccagcgtgggtgacagagtgaccatcacctgtagtgccagtcagagccttgagaacagcaacggaaacacctacctgaattggtaccagcagaagccaggtaaggctccaaagctgctgatctacagagtttccaaccgattctctggtgtgccaagcagattcagcggtagcggtagcggtaccgacttcaccctcaccatcagcagcctccagccagaggacttcgccacctactactgcctccagctgactcatgtcccatggaccttcggtcagggcaccaaggtggagatcaaacgc

SEQ ID NO: 13 - protein, 339 aa, Homo sapiens
  REGION 1..20: note = Signal peptide
  REGION 21..269: note = Extracellular domain
  REGION 270..339: note = Transmembrane and cytoplasmic domains
MSPSPTALFCLGLCLGRVPAQSGPLPKPSLQALPSSLVPLEKPVTLRCQGPPGVDLYRLEKLSSSRYQDQAVLFIPAMKRSLAGRYRCSYQNGSLWSLPSDQLELVATGVFAKPSLSAQPGPAVSSGGDVTLQCQTRYGFDQFALYKEGDPAPYKNPERWYRASFPIITVTAAHSGTYRCYSFSSRDPYLWSAPSDPLELVVTGTSVTPSRLPTEPPSSVAEFSEATAELTVSFTNKVFTTETSRSITTSPKESDSPAGPARQYYTKGNLVRICLGAVILIILAGFLAEDWHSRRKRLRHRGRAVQRPLPPLPPLPQTRKSHGGQDGGRQDVHSRGLCS

SEQ ID NO: 14 - DNA, 321 bp, synthetic construct
  source 1..321: mol_type = other DNA
  misc_feature 1..321: note = heavy chain constant region
gcctccaccaagggtccctcagtcttcccactggcaccctcctccaagagcacctctggtggcacagctgccctgggctgcctggtcaaggactacttcccagaaccagtgactgtgtcatggaactcaggcgccctgaccagcggcgtgcacaccttccctgctgtcttgcagtcctcaggactctactccctcagcagcgtggtgaccgtgccctccagcagcttgggcacccagacctacatctgcaacgtgaatcacaagcccagcaacaccaaggtggacaagaaagtcgagcctaagtcatgcgacaagactcac

SEQ ID NO: 15 - DNA, 318 bp, synthetic construct
  source 1..318: mol_type = other DNA
  misc_feature 1..318: note = light chain constant region
actgtggctgcaccaagtgtgttcatcttcccacctagcgatgagcagttgaaatctggaactgcctctgtcgtgtgcctcctgaacaacttctacccacgggaggccaaggtacagtggaaggtggataacgccctccaatccggtaactcccaggagagtgtcacagagcaagatagcaaggacagcacctacagcctcagcagcaccctgactctgagcaaagcagactacgagaagcacaaggtctacgcctgcgaagtcacccatcagggcctgagttcccctgtcacaaagagcttcaaccggggagagtgt

SEQ ID NO: 16 - DNA, 66 bp, synthetic construct
  source 1..66: mol_type = other DNA
  misc_feature 1..66: note = signal peptide
atggatatgcgtgtaccagctcaactacttggacttctattgctttggcttcgtggtgctagatgt

SEQ ID NO: 17 - DNA, 57 bp, synthetic construct
  source 1..57: mol_type = other DNA
  misc_feature 1..57: note = signal peptide
atggactggacttggagaatcctattcttggttgctgcagctacaggtgctcattca

SEQ ID NO: 18 - DNA, 762 bp, synthetic construct
  source 1..762: mol_type = other DNA
  misc_feature 1..762: note = vector
gcggccgccaccatggactggacttggagaatcctattcttggttgctgcagctacaggtgctcattcacaggttcagctggttcagtcaggggctgaggtgaagaagcctggagcctcagtgaaggtgtcctgcaaggcttctggctacacatttaccagttacaatatgcactgggtaagacaggctcctggacagggcctggaatggatgggaggtatttatccaggaaatggtgatacttcctacaatcagaagttccagggccgagttactatgactcgggacacttccacctctacagtgtacatggagctcagcagcctgagatctgaggacaccgcggtctattactgtgcaagaggcaccgtggtcggcgactggtacttcgatgtgtggggccaaggcaccctggtcaccgtgagcagtgcctccaccaagggtccctcagtcttcccactggcaccctcctccaagagcacctctggtggcacagctgccctgggctgcctggtcaaggactacttcccagaaccagtgactgtgtcatggaactcaggcgccctgaccagcggcgtgcacaccttccctgctgtcttgcagtcctcaggactctactccctcagcagcgtggtgaccgtgccctccagcagcttgggcacccagacctacatctgcaacgtgaatcacaagcccagcaacaccaaggtggacaagaaagtcgagcctaagtcatgcgacaagactcactgatgaggatcc

SEQ ID NO: 19 - DNA, 742 bp, synthetic construct
  source 1..742: mol_type = other DNA
  misc_feature 1..742: note = vector
gacgtcaccatggatatgcgtgtaccagctcaactacttggacttctattgctttggcttcgtggtgctagatgtgacatccagatgacccagagcccaagcagcctgagcgccagcgtgggtgacagagtgaccatcacctgtagaagtagtcagagccttgagaacagcaacggaaacacctacctgaattggtaccagcagaagccaggtaaggctccaaagctgctgatctacagagtttccaaccgattctctggtgtgccaagcagattcagcggtagcggtagcggtaccgacttcaccttcaccatcagcagcctccagccagaggacatcgccacctactactgcctccagctgactcatgtcccatggaccttcggtcagggcaccaaggtggagatcacccggactgtggctgcaccaagtgtgttcatcttcccacctagcgatgagcagttgaaatctggaactgcctctgtcgtgtgcctcctgaacaacttctacccacgggaggccaaggtacagtggaaggtggataacgccctccaatccggtaactcccaggagagtgtcacagagcaagatagcaaggacagcacctacagcctcagcagcaccctgactctgagcaaagcagactacgagaagcacaaggtctacgcctgcgaagtcacccatcagggcctgagttcccctgtcacaaagagcttcaaccggggagagtgttgatgatatc

SEQ ID NO: 20 - DNA, 742 bp, synthetic construct
  source 1..742: mol_type = other DNA
  misc_feature 1..742: note = vector
gacgtcaccatggatatgcgtgtaccagctcaactacttggacttctattgctttggcttcgtggtgctagatgtgacatccagatgacccagagcccaagcagcctgagcgccagcgtgggtgacagagtgaccatcacctgtagtgccagtcagagccttgagaacagcaacggaaacacctacctgaattggtaccagcagaagccaggtaaggctccaaagctgctgatctacagagtttccaaccgattctctggtgtgccaagcagattcagcggtagcggtagcggtaccgacttcaccctcaccatcagcagcctccagccagaggacttcgccacctactactgcctccagctgactcatgtcccatggaccttcggtcagggcaccaaggtggagatcaaacgcactgtggctgcaccaagtgtgttcatcttcccacctagcgatgagcagttgaaatctggaactgcctctgtcgtgtgcctcctgaacaacttctacccacgggaggccaaggtacagtggaaggtggataacgccctccaatccggtaactcccaggagagtgtcacagagcaagatagcaaggacagcacctacagcctcagcagcaccctgactctgagcaaagcagactacgagaagcacaaggtctacgcctgcgaagtcacccatcagggcctgagttcccctgtcacaaagagcttcaaccggggagagtgttgatgatatc

SEQ ID NO: 21 - protein, 5 aa, synthetic construct
  REGION 1..5: note = CDR-H2 - Residues before
LEWIG